European Patent Application EP 4 338 750 A2, published March 20, 2024. Title: Anti-CD40 Antibodies and Uses Thereof. Applicant: BETH ISRAEL DEACONESS MEDICAL CENTER, INC. Application EP, filed March 12, 2012. The sequence listing filed with the application follows.

SEQUENCE LISTING (10 sequences)

SEQ ID NO: 1 - DNA, 396 bp, synthetic construct
  source 1..396: mol_type = other DNA
atggaaaggcactggatctttctcttcctgttgtcagtaactgcaggtgtccactcccaggtccagctgcaacagtctggggctgaactggcaaaacctggggcctcagtgaagatgtcctgtaaggcttctggctacacctttactaactactggatgcactgggtaaaacagaggcctggacagggtctggaatggattggatacattaatcctagcaatgattatactaagtacaatcaaaagttcaaggacaaggccacattgactgcagacaaatcctccaacacagcctacatgcaactgggtagcctgacatctgaggactctgcagtctattattgtgcaagacaggggtttccttactggggccaagggactctggtcactgtctct

SEQ ID NO: 2 - protein, 132 aa, synthetic construct
MERHWIFLFLLSVTAGVHSQVQLQQSGAELAKPGASVKMSCKASGYTFTNYWMHWVKQRPGQGLEWIGYINPSNDYTKYNQKFKDKATLTADKSSNTAYMQLGSLTSEDSAVYYCARQGFPYWGQGTLVTVS

SEQ ID NO: 3 - DNA, 384 bp, synthetic construct
  source 1..384: mol_type = other DNA
atggattttcaagtgcagattttcagcttcctgctaatcagtgcctcagtcataatatccagaggacaaattgttctcacccagtctccagcaatcatgtctgcatctccaggggagaaggtcaccatgacctgcagtgccagctcaagtgtaagttacatgcactggtaccaccagaggtcaggcacctcccccaaaagatggatttatgacacatccaaactggcttctggagtccctgctcgcttcagtggcagtgggtctgggacctcttactctctcacaatcagcagcatggaggctgaagatgctgccacttattactgccaccagttgagtagtgacccattcacgttcggctcggggacaaagttggaaataaaa

SEQ ID NO: 4 - protein, 128 aa, synthetic construct
  REGION 1..128: note = Synthetic Construct
MDFQVQIFSFLLISASVIISRGQIVLTQSPAIMSASPGEKVTMTCSASSSVSYMHWYHQRSGTSPKRWIYDTSKLASGVPARFSGSGSGTSYSLTISSMEAEDAATYYCHQLSSDPFTFGSGTKLEIK

SEQ ID NO: 5 - protein, 100 aa, synthetic construct
EPPTACREKQYLINSQCCSLCQPGQKLVSDCTEFTETECLPCSESEFLDTWNRETRCHQHKYCDPNLGLRVQQKGTSETDTICTCEEGLHCMSESCESCV

SEQ ID NO: 6 - protein, 100 aa, synthetic construct
EPPTACREKQYLINSQCCSLCQPGQKLVSDCTEFTETECLPCGESEFLDTWNRETHCHQHKYCDPNLGLRVQQKGTSETDTICTCEEGWHCTSEACESCV

SEQ ID NO: 7 - DNA, 30 bp, synthetic construct
  source 1..30: mol_type = other DNA
ctaacactcattcctgttgaagctcttgac

SEQ ID NO: 8 - DNA, 24 bp, synthetic construct
  source 1..24: mol_type = other DNA
gctgatgctgcaccaactgtatcc

SEQ ID NO: 9 - DNA, 20 bp, synthetic construct
  source 1..20: mol_type = other DNA
ggcaacgttgcaggtctcgc

SEQ ID NO: 10 - DNA, 26 bp, synthetic construct
  source 1..26: mol_type = other DNA
ctggatctgctgcccaaactaactcc